European Patent Specification EP 3 711 776 B1, published January 11, 2023. Title: MODIFIED HOST CELLS AND USES THEREOF. Applicant: GlaxoSmithKline Biologicals S.A. GlycoVaxyn AG. Application TBA. The sequence listing filed with the application follows.

SEQUENCE LISTING (3 sequences)

SEQ ID NO: 1 - protein, 5 aa, Artificial Sequence
  N-Glycosylation Consensus Sequence
  MISC_FEATURE (1)..(1): Xaa = Asp or Glu
  MISC_FEATURE (2)..(2): Xaa = any natural amino acid except Pro
  MISC_FEATURE (4)..(4): Xaa = any natural amino acid except Pro
  MISC_FEATURE (5)..(5): Xaa = Ser or Thr
XXNXX

SEQ ID NO: 2 - protein, 558 aa, Pseudomonas aeruginosa O6
  formyltransferase
MSWQLFSEKCRFLGAVEISQHFWGFIVLEASFGMKIKAALIVDDLSLSEWQKRAIEDSSEYLDIQLVLSCRNSATKKSVIKHCGYYFLNILSLKNDMTRRVQLDSRGSEVIHFDSDYEGAWQRIPEDVCARILDKGIKLVIKFGMSLLRIDGGLQRLDILSYHHGDPEYYRGRPAGFYEIYENADSVGIIVQKLSNKLDAGEVLVRGYSKVHHHSYKKTSRNFYLNSVVLLRKALVNYSRGEQVVLEKLGKNYRLPSNFTVFKFFCKTIFRGLARLSYGAFFEKKWNVVALPYNDIPSLQELSVSAGKIPKVEKGYTFYADPFFSADGKLIRLEALNASNGLGEIIELKAQSLDFSRVILKGNHFSYPYSFEASGVEYLIPEVASHSAPCLLPPPFALESKKLFQGMEGERILDGTLFEHGGRYYLFCGQAVSGSDNLYLYVGESLEGPYTSHPCNPVVMNPGSARMGGRIFKEGGKLYRFGQNNSYGYGSSLAVNEIEVLDPEHYSEKRVANLAFQDARGPHTIDIHGQTMILDFYQDRFSLLAGYRRLVARLLSRG

SEQ ID NO: 3 - protein, 417 aa, Pseudomonas aeruginosa O6
  wzy polymerase
MYAMLTGATLLIFAVAARLLARSAIHPSVAMPITWGLGLIGVSLASLIGFYRVESDALLIFLFGVMSFSLSAGCFSFLYNGYFRAPSSNFLFDSELRTRALVIFFCLAHIVFLTVIYRDLSSIAPTLREAAYMARAQSVSGEPVLSSLSMNYLQLGQTVIPLVVLLYLRGKCGVLGFLAISVPWMGVILLASGRASLMQMLVGLFFIYILVKGSPSLKSLLVIGLAMFLVIAVGAVATSKIQFHEGDGISTLFIELYRHVAGYALQGPVLFDRYYQGSIHLEPYWSPLNGFCSILATVGLCQKPPLHLDFYEYAPGELGNVYSMFFSMYPHYGALGVIGVMALYGMLCSYAYCKAKKGSLYFTVLSSYLFSAIVFSLFSDQISTSWWFYVKMTIILGILCFVFRRDRMFVIRLPQAG